European Patent Application EP 4 234 715 A1, published August 30, 2023. Title: METHOD FOR TESTING TARGET NUCLEIC ACID IN SAMPLE. Applicant: BEIJING SYNSORTECH CO., LTD. ZHEJIANG SYNSORBIO TECHNOLOGY CO., LTD. BEIJING SYNSORBIO TECHNOLOGY CO., LTD. Application PCT/CN2021/118280. The sequence listing filed with the application follows.

SEQUENCE LISTING (6 sequences)

SEQ ID NO: 1 - RNA, 105 nt, Artificial sequence
  Description of artificial sequence: synthetic sequence
gucuaaaggacagaauuuuucaacgggugugccaauggccacuuuccagguggcaaagcccguugaacuucaagcgaaguggcacacucaauacuugagcacacu

SEQ ID NO: 2 - DNA, 34 bp, Artificial sequence
  Description of artificial sequence: synthetic sequence
gttgtagcttgtcacaccgtttctatagattagc

SEQ ID NO: 3 - DNA, 32 bp, Artificial sequence
  Description of artificial sequence: synthetic sequence
cctggtttaacatatagtgaaccgccacacat

SEQ ID NO: 4 - RNA, 105 nt, Artificial sequence
  Description of artificial sequence: synthetic sequence
gaguccuuugggcuuccaggcaacgggugugccaauggccacuuuccagguggcaaagcccguugaacuucaagcgaaguggcacacucaauacuugagcacacu

SEQ ID NO: 5 - DNA, 35 bp, Artificial sequence
  Synthetic sequence
tgagtactggacctcggaccagagccatgtaagaa

SEQ ID NO: 6 - DNA, 35 bp, Artificial sequence
  Description of artificial sequence: synthetic sequence
gcccaccaagagacaattacccccaccctcaatgc